European Patent Specification EP 3 759 216 B1, published April 12, 2023. Title: TRANSDUCTION AND EXPANSION OF CELLS. Applicant: Imperial Innovations Limited. The sequence listing filed with the application follows.

SEQUENCE LISTING (12 sequences)

SEQ ID NO: 1 - DNA, 20 bp, Artificial Sequence
  CD1D primer
ccctgagaaagtgaccttgg

SEQ ID NO: 2 - DNA, 21 bp, Artificial Sequence
  CD1D primer
tggctgttagctttcagttcc

SEQ ID NO: 3 - DNA, 20 bp, Artificial Sequence
  GAPDH primer
ccgggagaagctgagtcatg

SEQ ID NO: 4 - DNA, 20 bp, Artificial Sequence
  GAPDH primer
tttgcggtggaaatgtcctt

SEQ ID NO: 5 - DNA, 22 bp, Artificial Sequence
  HOXA2 primer
aggaaagattttggttgggaag

SEQ ID NO: 6 - DNA, 22 bp, Artificial Sequence
  HOXA2 primer
aaaaagagggaaagggacagac

SEQ ID NO: 7 - DNA, 21 bp, Artificial Sequence
  Distal primer
tggacgtccgagaggtaagag

SEQ ID NO: 8 - DNA, 23 bp, Artificial Sequence
  Distal primer
cacagtaacctggagatccacta

SEQ ID NO: 9 - DNA, 20 bp, Artificial Sequence
  Proximal primer
aatgatgctggggtgtgagg

SEQ ID NO: 10 - DNA, 20 bp, Artificial Sequence
  Proximal primer
gcacggcctgcaagattatg

SEQ ID NO: 11 - DNA, 20 bp, Artificial Sequence
  Region within exon 2 at +382 primer
ctccagatctcgtccttcgc

SEQ ID NO: 12 - DNA, 20 bp, Artificial Sequence
  Region within exon 2 at +382 primer
ctgggaccaaggcttcagag